European Patent Application EP 4 159 839 A1, published April 5, 2023. Title: Antiviral agent. Applicant: TOHOKU UNIVERSITY. The sequence listing filed with the application follows.

SEQUENCE LISTING (60 sequences)

SEQ ID NO: 1 - DNA, 1487 bp, Lactobacillus sp.
  misc_feature: Inventor:KITAZAWA, Haruki; ASO, Hisashi; OHTSUBO, Wakako
  misc_feature: 16S rRNA of the present Lactobacillus bacteria strain
gacgaacgctggcggcgtgcctaatacatgcaagtcgaacgaaactttcttacaccgaatgcttgcattcaccgtaagaagttgagtggcggacgggtgagtaacacgtgggtaacctgcctaaaagaaggggataacacttggaaacaggtgctaataccgtatatctctaaggatcgcatgatccttagatgaaagatggttctgctatcgcttttagatggacccgcggcgtattaactagttggtggggtaacggcctaccaaggtgatgatacgtagccgaactgagaggttgatcggccacattgggactgagacacggcccaaactcctacgggaggcagcagtagggaatcttccacaatggacgcaagtctgatggagcaacgccgcgtgagtgaagaaggtcttcggatcgtaaaactctgttgttagagaagaacacgagtgagagtaactgttcattcgatgacggtatctaaccagcaagtcacggctaactacgtgccagcagccgcggtaatacgtaggtggcaagcgttgtccggatttattgggcgtaaagggaacgcaggcggtcttttaagtctgatgtgaaagccttcggcttaaccggagtagtgcattggaaactggaagacttgagtgcagaagaggagagtggaactccatgtgtagcggtgaaatgcgtagatatatggaagaacaccagtggcgaaagcggctctctggtctgtaactgacgctgaggttcgaaagcgtgggtagcaaacaggattagataccctggtagtccacgccgtaaacgatgaatgctaggtgttggagggtttccgcccttcagtgccgcagctaacgcaataagcattccgcctggggagtacgaccgcaaggttgaaactcaaaggaattgacgggggcccgcacaagcggtggagcatgtggtttaattcgaagcaacgcgaagaaccttaccaggtcttgacatcctttgaccacctaagagattaggttttcccttcggggacaaagtgacaggtggtgcatggctgtcgtcagctcgtgtcgtgagatgttgggttaagtcccgcaacgagcgcaacccttgttgtcagttgccagcattaagttgggcactctggcgagactgccggtgacaaaccggaggaaggtggggacgacgtcaagtcatcatgccccttatgacctgggctacacacgtgctacaatggacggtacaacgagtcgcgagaccgcgaggtttagctaatctcttaaagccgttctcagttcggattgtaggctgcaactcgcctacatgaagtcggaatcgctagtaatcgcgaatcagcatgtcgcggtgaatacgttcccgggccttgtacacaccgcccgtcacaccatgagagtttgtaacacccaaagccggtggggtaaccgcaaggagccagccgtctaaggtgggacagatgattggggtgaag

SEQ ID NO: 2 - DNA, 20 bp, Artificial
  À-actin sense primer
tggataagctgcagtcacag

SEQ ID NO: 3 - DNA, 22 bp, Artificial
  À-actin antisense primer
gcgtagaggtcctccctgatgt

SEQ ID NO: 4 - DNA, 20 bp, Artificial
  IFN- À sense primer
agttgcctgggactcctcaa

SEQ ID NO: 5 - DNA, 22 bp, Artificial
  IFN- À antisense primer
cctcagggacctcaaagttcat

SEQ ID NO: 6 - DNA, 25 bp, Artificial
  IFN- É sense primer
ccttagaggctgagctagacttgac

SEQ ID NO: 7 - DNA, 22 bp, Artificial
  IFN- É antisense primer
agcctgaagttcgacgtggatg

SEQ ID NO: 8 - DNA, 18 bp, Artificial
  Mx1 sense primer
gaggtggaccccgaagga

SEQ ID NO: 9 - DNA, 18 bp, Artificial
  Mx1 antisense primer
caccagatccggcttcgt

SEQ ID NO: 10 - DNA, 20 bp, Artificial
  OAS1 sense primer
ccaacaggttcagacagcct

SEQ ID NO: 11 - DNA, 20 bp, Artificial
  OAS1 antisense primer
gaggagccacccttcacaac

SEQ ID NO: 12 - DNA, 18 bp, Artificial
  RNaseL sense primer
gcagccgagccaacgata

SEQ ID NO: 13 - DNA, 19 bp, Artificial
  RNaseL antisense primer
agctcccgtcgctctcact

SEQ ID NO: 14 - DNA, 20 bp, Artificial
  PKR sense primer
ccctgcacttctagccatct

SEQ ID NO: 15 - DNA, 21 bp, Artificial
  PKR antisense primer
cgaccactggccatttctttc

SEQ ID NO: 16 - DNA, 20 bp, Artificial
  RIG-I sense primer
tatccgagcagcaggctttg

SEQ ID NO: 17 - DNA, 22 bp, Artificial
  RIG-I antisense primer
ctcgttgctgggatctatggcc

SEQ ID NO: 18 - DNA, 20 bp, Artificial
  TLR2 sense primer
acatgaagatgatgtgggcc

SEQ ID NO: 19 - DNA, 20 bp, Artificial
  TLR2 antisense primer
taggagtcctgctcactgta

SEQ ID NO: 20 - DNA, 20 bp, Artificial
  TLR3 sense primer
tagagacatggattgctccc

SEQ ID NO: 21 - DNA, 20 bp, Artificial
  TLR3 antisense primer
aacttctggaatgcaggtcc

SEQ ID NO: 22 - DNA, 20 bp, Artificial
  TLR4 sense primer
ctctgccttcactacagaga

SEQ ID NO: 23 - DNA, 20 bp, Artificial
  TLR4 antisense primer
ctctgccttcactacagaga

SEQ ID NO: 24 - DNA, 20 bp, Artificial
  NOD1 sense primer
ctgtcgtcaacaccgatcca

SEQ ID NO: 25 - DNA, 19 bp, Artificial
  NOD1 antisense primer
ccagttggtgacgcagctt

SEQ ID NO: 26 - DNA, 22 bp, Artificial
  NOD2 sense primer
gagcgcatcctcttaactttcg

SEQ ID NO: 27 - DNA, 19 bp, Artificial
  NOD2 antisense primer
acgctcgtgatccgtgaac

SEQ ID NO: 28 - DNA, 22 bp, Artificial
  MCP-1 sense primer
acagaagagtcaccagcagcaa

SEQ ID NO: 29 - DNA, 16 bp, Artificial
  MCP-1 antisense primer
gcccgcgatggtcttg

SEQ ID NO: 30 - DNA, 20 bp, Artificial
  IL-6 sense primer
tccataagctgcagtcacag

SEQ ID NO: 31 - DNA, 20 bp, Artificial
  IL-6 antisense primer
attatccgaatggccctcag

SEQ ID NO: 32 - DNA, 21 bp, Artificial
  IL-8 sense primer
gctctctgtgaggctgcagtt

SEQ ID NO: 33 - DNA, 22 bp, Artificial
  IL-8 antisense primer
tttatgcactggcatcgaagtt

SEQ ID NO: 34 - DNA, 20 bp, Artificial
  IL-12 sense primer
agttccaggccatgaatgca

SEQ ID NO: 35 - DNA, 20 bp, Artificial
  IL-12 antisense primer
tggcacagtctcactgttga

SEQ ID NO: 36 - DNA, 24 bp, Artificial
  IL-18 sense primer
tgaaccggaagacaattgcatcag

SEQ ID NO: 37 - DNA, 25 bp, Artificial
  IL-18 antisense primer
ccaggtcttcatcgttttcagctac

SEQ ID NO: 38 - DNA, 20 bp, Artificial
  TNF ¿ sense primer
cgactcagtgccgagatcaa

SEQ ID NO: 39 - DNA, 20 bp, Artificial
  TNF ¿ antisense primer
cctgcccagattcagcaaag

SEQ ID NO: 40 - DNA, 19 bp, Artificial
  A20 sense primer
cctccctggaaagccagaa

SEQ ID NO: 41 - DNA, 21 bp, Artificial
  A20 antisense primer
gtgccacaagcttcctcactt

SEQ ID NO: 42 - DNA, 19 bp, Artificial
  BCL-3 sense primer
cgacgcggtggacattaag

SEQ ID NO: 43 - DNA, 23 bp, Artificial
  BCL-3 antisense primer
accatgctaaggctgttgttttc

SEQ ID NO: 44 - DNA, 17 bp, Artificial
  Tollip sense primer
taccgtgggccgtctca

SEQ ID NO: 45 - DNA, 21 bp, Artificial
  Tollip antisense primer
ccgtagttcttcgccaacttg

SEQ ID NO: 46 - DNA, 20 bp, Artificial
  IRAK-M sense primer
tggagcagccttgaatcctt

SEQ ID NO: 47 - DNA, 23 bp, Artificial
  IRAK-M antisense primer
tggataacacgtttgggaatctt

SEQ ID NO: 48 - DNA, 20 bp, Artificial
  MKP-1 sense primer
aacgagggtcaggcttttcc

SEQ ID NO: 49 - DNA, 21 bp, Artificial
  MKP-1 antisense primer
tccccaatgtgctgagttcag

SEQ ID NO: 50 - DNA, 22 bp, Artificial
  SIGIRR sense primer
atgtgaagtgtcggctcaatgt

SEQ ID NO: 51 - DNA, 22 bp, Artificial
  SIGIRR antisense primer
ttcatctccacctccccatact

SEQ ID NO: 52 - DNA, 1492 bp, Lactobacillus sp.
  misc_feature: 16S rRNA of the present Lactobacillus bacteria strain #16
gacgaacgctggcggcgtgcctaatacatgcaagtcgaacgaactctggtaatgattggtgcttgcatcatgaattacatttgagtgagtggcgaactggtgagtaacacgtgggaaacctgcccagaagcgggggataacacctggaaacagatgctaataccgcataacaacttggaccgcatggtccgagtttgaaagatggcttcggctatcacttttggatggtcccgcggcgtattagctagatggtgaggtaacggctcaccatggcaatgatacgtagccgacctgagagggtaatcggccacattgggactgagacacggcccaaactcctacgggaggcagcagtagggaatcttccacaatggacgaaagtctgatggagcaacgccgcgtgagtgaagaagggtttcggctcgtaaaactctgttgttaaagaagaacatatctgagagtaactgttcaggtattgacggtatttaaccagaaagccacggctaactacgtgccagcagccgcggtaatacgtaggtggcaagcgttgtccggatttattgggcgtaaagcgagcgcaggcggttttttaagtctgatgtgaaagccttcggctcaaccgaagaagtgcatcggaaactgggraacttgagtgcagaagaggacagtggaactccatgtgtagcggtgaaatgcgtagatatatggaagaacaccagtggcgaaggcggctgtctggtctgtaactgacgctgaggctcgaaagtatgggtagcaaacaggattagataccctggtagtccataccgtaaacgatgaatgctaagtgttggagggtttccgcccttcagtgctgcagctaacgcattaagcattccgcctggggagtacggccgcaaggctgaaactcaaaggaattgacgggggcccgcacaagcggtggagcatgtggtttaattcgaagctacgcgaagaaccttaccaggtcttgacatactatgcaaatctaagagattagacgttcccttcggggacatggatacaggtggtgcatggttgtcgtcagctcgtgtcgtgagatgttgggttaagtcccgcaacgagcgcaacccttattatcagttgccagcattaagttgggcactctggtgagactgccggtgacaaaccggaggaaggtggggatgacgtcaaatcatcatgccccttatgacctgggctacacacgtgctacaatggatggtacaacgagttgcgaactcgcgagagtaagctaatctcttaaagccattctcagttcggattgtaggctgcaactcgcctacatgaagtcggaatcgctagtaatcgcggatcagcatgccgcggtgaatacgttcccgggccttgtacacaccgcccgtcacaccatgagagtttgtaacacccaaagtcggtggggtaaccttttaggaaccagccgcctaaggtgggacagatgattagggtgaag

SEQ ID NO: 53 - DNA, 1492 bp, Lactobacillus sp.
  misc_feature: 16S rRNA of the present Lactobacillus bacteria strain #6ML686 and #6ML6109
gacgaacgctggcggcgtgcctaatacatgcaagtcgaacgaactctggtattgattggtgcttgcatcatgatttacatttgagtgagtggcgaactggtgagtaacacgtgggaaacctgcccagaagcgggggataacacctggaaacagatgctaataccgcataacaacttggaccgcatggtccgagtttgaaagatggcttcggctatcacttytggatggtcccgcggcgtattagctagatggtgaggtaacggctcaccatggcaatgatacgtagccgacctgagagggtaatcggccacattgggactgagacacggcccaaactcctacgggaggcagcagtagggaatcttccacaatggacgaaagtctgatggagcaacgccgcgtgagtgaagaagggtttcggctcgtaaaactctgttgttaaagaagaacatatctgagagtaactgttcaggtattgacggtatttaaccagaaagccacggctaactacgtgccagcagccgcggtaatacgtaggtggcaagcgttgtccggatttattgggcgtaaagcgagcgcaggcggttttttaagtctgatgtgaaagccttcggctcaaccgaagaagtgcatcggaaactgggaaacttgagtgcagaagaggacagtggaactccatgtgtagcggtgaaatgcgtagatatatggaagaacaccagtggcgaaggcggctgtctggtctgtaactgacgctgaggctcgaaagtatgggtagcaaacaggattagataccctggtagtccataccgtaaacgatgaatgctaagtgttggagggtttccgcccttcagtgctgcagctaacgcattaagcattccgcctggggagtacggccgcaaggctgaaactcaaaggaattgacgggggcccgcacaagcggtggagcatgtggtttaattcgaagctacgcgaagaaccttaccaggtcttgacatactatgcaaatctaagagattagacgttcccttcggggacatggatacaggtggtgcatggttgtcgtcagctcgtgtcgtgagatgttgggttaagtcccgcaacgagcgcaacccttattatcagttgccagcattaagttgggcactctggtgagactgccggtgacaaaccggaggaaggtggggatgacgtcaaatcatcatgccccttatgacctgggctacacacgtgctacaatggatggtacaacgagttgcgaactcgcgagagtaagctaatctcttaaagccattctcagttcggattgtaggctgcaactcgcctacatgaagtcggaatcgctagtaatcgcggatcagcatgccgcggtgaatacgttcccgggccttgtacacaccgcccgtcacaccatgagagtttgtaacacccaaagtcggtggggtaaccttttaggaaccagccgcctaaggtgggacagatgattagggtgaag

SEQ ID NO: 54 - DNA, 1492 bp, Lactobacillus sp.
  misc_feature: 16S rRNA of the present Lactobacillus bacteria strain #6VG132
gacgaacgctggcggcgtgcctaatacatgcaagtcgaacgaactctggtattgattggtgcttgcatcatgatttacatttgagtgagtggcgaactggtgagtaacacgtgggaaacctgcccagaagcgggggataacacctggaaacagatgctaataccgcataacaacttggaccgcatggtccgagyttgaaagatggcttcggctatcacttttggatggtcccgcggcgtattagctagatggtgrggtaacggctcaccatggcaatgatacgtagccgacctgagagggtaatcggccacattgggactgagacacggcccaaactcctacgggaggcagcagtagggaatcttccacaatggacgaaagtctgatggagcaacgccgcgtgagtgaagaagggtttcggctcgtaaaactctgttgttaaagaagaacatatctgagagtaactgttcaggtattgacggtatttaaccagaaagccacggctaactacgtgccagcagccgcggtaatacgtaggtggcaagcgttgtccggatttattgggcgtaaagcgagcgcaggcggttttttaagtctgatgtgaaagccttcggctcaaccgaagaagtgcatcggaaactgggaaacttgagtgcagaagaggacagtggaactccatgtgtagcggtgaaatgcgtagatatatggaagaacaccagtggcgaaggcggctgtctggtctgtaactgacgctgaggctcgaaagtatgggtagcaaacaggattagataccctggtagtccataccgtaaacgatgaatgctaagtgttggagggtttccgcccttcagtgctgcagctaacgcattaagcattccgcctggggagtacggccgcaaggctgaaactcaaaggaattgacgggggcccgcacaagcggtggagcatgtggtttaattcgaagctacgcgaagaaccttaccaggtcttgacatactatgcaaatctaagagattagacgttcccttcggggacatggatacaggtggtgcatggttgtcgtcagctcgtgtcgtgagatgttgggttaagtcccgcaacgagcgcaacccttattatcagttgccagcattaagttgggcactctggtgagactgccggtgacaaaccggaggaaggtggggatgacgtcaaatcatcatgccccttatgacctgggctacacacgtgctacaatggatggtacaacgagttgcgaactcgcgagagtaagctaatctcttaaagccattctcagttcggattgtaggctgcaactcgcctacatgaagtcggaatcgctagtaatcgcggatcagcatgccgcggtgaatacgttcccgggccttgtacacaccgcccgtcacaccatgagagtttgtaacacccaaagtcggtggggtaaccttttaggaaccagccgcctaaggtgggacagatgattagggtgaag

SEQ ID NO: 55 - DNA, 1492 bp, Lactobacillus sp.
  misc_feature: 16S rRNA of the present Lactobacillus bacteria strain #6VG141
gacgaacgctggcggcgtgcctaatacatgcaagtcgaacgaactctggtattgattggtgcttgcatcatgatttacatttgagtgagtggcgaactggtgagtaacacgtgggaaacctgcccagaagcgggggataacacctggaaacagatgctaataccgcataacaacttggaccgcatggtccgagtttgaaagatggcttcggctatcacttctggatggtcccgcggcgtattagctagatggtgaggtaacggctcaccatggcaatgatacgtagccgacctgagagggtaatcggccacattgggactgagacacggcccaaactcctacgggaggcagcagtagggaatcttccacaatggacgaaagtctgatggagcaacgccgcgtgagtgaagaagggtttcggctcgtaaaactctgttgttaaagaagaacatatctgagagtaactgttcaggtattgacggtatttaaccagaaagccacggctaactacgtgccagcagccgcggtaatacgtaggtggcaagcgttgtccggatttattgggcgtaaagcgagcgcaggcggttttttaagtctgatgtgaaagccttcggctcaaccgaagaagtgcatcggaaactgggaaacttgagtgcagaagaggacagtggaactccatgtgtagcggtgaaatgcgtagatatatggaagaacaccagtggcgaaggcggctgtctggtctgtaactgacgctgaggctcgaaagtatgggtagcaaacaggattagataccctggtagtccataccgtaaacgatgaatgctaagtgttggagggtttccgcccttcagtgctgcagctaacgcattaagcattccgcctggggagtacggccgcaaggctgaaactcaaaggaattgacgggggcccgcacaagcggtggagcatgtggtttaattcgaagctacgcgaagaaccttaccaggtcttgacatactatgcaaatctaagagattagacgttcccttcggggacatggatacaggtggtgcatggttgtcgtcagctcgtgtcgtgagatgttgggttaagtcccgcaacgagcgcaacccttattatcagttgccagcattaagttgggcactctggtgagactgccggtgacaaaccggaggaaggtggggatgacgtcaaatcatcatgccccttatgacctgggctacacacgtgctacaatggatggtacaacgagttgcgaactcgcgagagtaagctaatctcttaaagccattctcagttcggattgtaggctgcaactcgcctacatgaagtcggaatcgctagtaatcgcggatcagcatgccgcggtgaatacgttcccgggccttgtacacaccgcccgtcacaccatgagagtttgtaacacccaaagtcggtggggtaaccttttaggaaccagccgcctaaggtgggacagatgattagggtgaag

SEQ ID NO: 56 - DNA, 1492 bp, Lactobacillus sp.
  misc_feature: 16S rRNA of the present Lactobacillus bacteria strain #2CS82 and #1FeB18
gacgaacgctggcggcgtgcctaatacatgcaagtcgaacgaactctggtattgattggtgcttgcatcatgatttacatttgagtgagtggcgaactggtgagtaacacgtgggaaacctgcccagaagcgggggataacacctggaaacagatgctaataccgcataacaacttggaccgcatggtccgagcttgaaagatggcttcggctatcacttttggatggtcccgcggcgtattagctagatggtggggtaacggctcaccatggcaatgatacgtagccgacctgagagggtaatcggccacattgggactgagacacggcccaaactcctacgggaggcagcagtagggaatcttccacaatggacgaaagtctgatggagcaacgccgcgtgagtgaagaagggtttcggctcgtaaaactctgttgttaaagaagaacatatctgagagtaactgttcaggtattgacggtatttaaccagaaagccacggctaactacgtgccagcagccgcggtaatacgtaggtggcaagcgttgtccggatttattgggcgtaaagcgagcgcaggcggttttttaagtctgatgtgaaagccttcggctcaaccgaagaagtgcatcggaaactgggaaacttgagtgcagaagaggacagtggaactccatgtgtagcggtgaaatgcgtagatatatggaagaacaccagtggcgaaggcggctgtctggtctgtaactgacgctgaggctcgaaagtatgggtagcaaacaggattagataccctggtagtccataccgtaaacgatgaatgctaagtgttggagggtttccgcccttcagtgctgcagctaacgcattaagcattccgcctggggagtacggccgcaaggctgaaactcaaaggaattgacgggggcccgcacaagcggtggagcatgtggtttaattcgaagctacgcgaagaaccttaccaggtcttgacatactatgcaaatctaagagattagacgttcccttcggggacatggatacaggtggtgcatggttgtcgtcagctcgtgtcgtgagatgttgggttaagtcccgcaacgagcgcaacccttattatcagttgccagcattaagttgggcactctggtgagactgccggtgacaaaccggaggaaggtggggatgacgtcaaatcatcatgccccttatgacctgggctacacacgtgctacaatggatggtacaacgagttgcgaactcgcgagagtaagctaatctcttaaagccattctcagttcggattgtaggctgcaactcgcctacatgaagtcggaatcgctagtaatcgcggatcagcatgccgcggtgaatacgttcccgggccttgtacacaccgcccgtcacaccatgagagtttgtaacacccaaagtcggtggggtaaccttttaggaaccagccgcctaaggtgggacagatgattagggtgaag

SEQ ID NO: 57 - DNA, 1492 bp, Lactobacillus sp.
  misc_feature: 16S rRNA of the present Lactobacillus bacteria strain #3CS123
gacgaacgctggcggcgtgcctaatacatgcaagtcgaacgaactctggtattgattggtgcttgcatcatgatttacatttgagtgagtggcgaactggtgagtaacacgtgggaaacctgcccagaagcgggggataacacctggaaacagatgctaataccgcataacaacttggaccgcatggtccgagtttgaaagatggcttcggctatcacttttggatggtcccgcggcgtattagctagatggtgrggtaacggctcaccatggcaatgatacgtagccgacctgagagggtaatcggccacattgggactgagacacggcccaaactcctacgggaggcagcagtagggaatcttccacaatggacgaaagtctgatggagcaacgccgcgtgagtgaagaagggtttcggctcgtaaaactctgttgttaaagaagaacatatctgagagtaactgttcaggtattgacggtatttaaccagaaagccacggctaactacgtgccagcagccgcggtaatacgtaggtggcaagcgttgtccggatttattgggcgtaaagcgagcgcaggcggttttttaagtctgatgtgaaagccttcggctcaaccgaagaagtgcatcggaaactgggaaacttgagtgcagaagaggacagtggaactccatgtgtagcggtgaaatgcgtagatatatggaagaacaccagtggcgaaggcggctgtctggtctgtaactgacgctgaggctcgaaagtatgggtagcaaacaggattagataccctggtagtccataccgtaaacgatgaatgctaagtgttggagggtttccgcccttcagtgctgcagctaacgcattaagcattccgcctggggagtacggccgcaaggctgaaactcaaaggaattgacgggggcccgcacaagcggtggagcatgtggtttaattcgaagctacgcgaagaaccttaccaggtcttgacatactatgcaaatctaagagattagacgttcccttcggggacatggatacaggtggtgcatggttgtcgtcagctcgtgtcgtgagatgttgggttaagtcccgcaacgagcgcaacccttattatcagttgccagcattaagttgggcactctggtgagactgccggtgacaaaccggaggaaggtggggatgacgtcaaatcatcatgccccttatgacctgggctacacacgtgctacaatggatggtacaacgagttgcgaactcgcgagagtaagctaatctcttaaagccattctcagttcggattgtaggctgcaactcgcctacatgaagtcggaatcgctagtaatcgcggatcagcatgccgcggtgaatacgttcccgggccttgtacacaccgcccgtcacaccatgagagtttgtaacacccaaagtcggtggggtaaccttttaggaaccagccgcctaaggtgggacagatgattagggtgaag

SEQ ID NO: 58 - DNA, 1502 bp, Lactobacillus sp.
  misc_feature: 16S rRNA of the present Lactobacillus bacteria strain #4FeB195
gatgaacgccggcggtgtgcctaatacatgcaagtcgaacgcgttggcccaactgattgaacgtgcttgcacggacttgacgttggtttaccagcgagtggcggacgggtgagtaacacgtaggtaacctgccccaaagcgggggataacatttggaaacagatgctaataccgcataacaatttgaatcgcatgattcaaatttaaaagatggcttcggctatcactttgggatggacctgcggcgcattagcttgttggtagggtaacggcctaccaaggctgtgatgcgtagccgagttgagagactgatcggccacaatggaactgagacacggtccatactcctacgggaggcagcagtagggaatcttccacaatgggcgcaagcctgatggagcaacaccgcgtgagtgaagaagggtttcggctcgtaaagctctgttgttagagaagaacgtgcgtgagagcaactgttcacgcagtgacggtatctaaccagaaagtcacggctaactacgtgccagcagccgcggtaatacgtaggtggcaagcgttatccggatttattgggcgtaaagcgagcgcaggcggtttgataagtctgatgtgaaagcctttggcttaaccaaagaagtgcatcggaaactgtcagacttgagtgcagaagaggacagtggaactccatgtgtagcggtggaatgcgtagatatatggaagaacaccagtggcgaaggcggctgtctggtctgcaactgacgctgaggctcgaaagcatgggtagcgaacaggattagataccctggtagtccatgccgtaaacgatgagtgctaggtgttggagggtttccgcccttcagtgccgcagctaacgcattaagcactccgcctggggagtacgaccgcaaggttgaaactcaaaggaattgacgggggcccgcacaagcggtggagcatgtggtttaattcgaagctacgcgaagaaccttaccaggtcttgacatcttgcgccaaccctagagatagggcgtttccttcgggaacgcaatgacaggtggtgcatggtcgtcgtcagctcgtgtcgtgagatgttgggttaagtcccgcaacgagcgcaacccttgttactagttgccagcattcagttgggcactctagtgagactgccggtgacaaaccggaggaaggtggggacgacgtcagatcatcatgccccttatgacctgggctacacacgtgctacaatggacggtacaacgagtcgcgaactcgcgagggcaagctaatctcttaaaaccgttctcagttcggactgcaggctgcaactcgcctgcacgaagtcggaatcgctagtaatcgcggatcagcatgccgcggtgaatacgttcccgggccttgtacacaccgcccgtcacaccatgagagtttgcaacacccaaagtcggtggggtaacccttcggggagctagccgcctaaggtggggcagatgattagggtgaag

SEQ ID NO: 59 - DNA, 25 bp, Artificial
  NSP5 sense primer
ctctttctggaaaatctattggtag

SEQ ID NO: 60 - DNA, 22 bp, Artificial
  NSP5 antisense primer
gatgaatccatagacacgccag